European Patent Specification EP 3 534 939 B1, published February 22, 2023. Title: VACCINE AGAINST PORCINE PARVOVIRUS AND. Applicant: Boehringer Ingelheim Vetmedica GmbH. The sequence listing filed with the application follows.

SEQUENCE LISTING (18 sequences)

SEQ ID NO: 1 - protein, 579 aa, Porcine parvovirus
MSENVEQHNPINAGTELSATGNESGGGGGGGGGRGAGGVGVSTGSFNNQTEFQYLGEGLVRITAHASRLIHLNMPEHETYKRIHVLNSESGVAGQMVQDDAHTQMVTPWSLIDANAWGVWFNPADWQLISNNMTEINLVSFEQEIFNVVLKTITESATSPPTKIYNNDLTASLMVALDTNNTLPYTPAAPRSETLGFYPWLPTKPTQYRYYLSCTRNLNPPTYTGQSEQITDSIQTGLHSDIMFYTIENAVPIHLLRTGDEFSTGIYHFDTKPLKLTHSWQTNRSLGLPPKLLTEPTTEGDQHPGTLPAANTRKGYHQTINNSYTEATAIRPAQVGYNTPYMNFEYSNGGPFLTPIVPTADTQYNDDEPNGAIRFTMGYQHGQLTTSSQELERYTFNPQSKCGRAPKQQFNQQSPLNLQNTNNGTLLPSDPIGGKTNMHFMNTLNTYGPLTALNNTAPVFPNGQIWDKELDTDLKPRLHVTAPFVCKNNPPGQLFVKIAPNLTDDFNADSPQQPRIITYSNFWWKGTLTFTAKMRSSNMWNPIQQHTTTAENIGNYIPTNIGGIKMFPEYSQLIPRKLY

SEQ ID NO: 2 - protein, 579 aa, Porcine parvovirus
MSENVEQHNPINAGTELSATGNESIGGGGGGGGRGSIGVGVSTGSFNNQTEFQYLGEGLVRITAHASRLIHLNMPEHETYKRIHVLNSESGVAGQMVQDDAHTQMVTPWSLIDANAWGVWFNPADWQLISNNMTEINLVSFEQEIFNVVLKTITESATSPPTKIYNNDLTASLMVALDTNNTLPYTPAAPRSETLGFYPWLPTKPTQYRYYLSCTRNLNPPTYTGQSEQITDSIQTGLHSDIMFYTIENAVPIHLLRTGDEFSTGIYHFDTKPLKLTHSWQTNRSLGLPPKLLTEPTTEGDQHPGTLPAANTRKGYHQTINNSYTEATAIRPAQVGYNTPYMNFEYSNGGPFLTPIVPTADTQYNDDEPNGAIRFTMGYQHGQLTTSSQELERYTFNPQSKCGRAPKQQFNQQSPLNLQNTNNGTLLPSDPIGGKTNMHFMNTLNTYGPLTALNNTAPVFPNGQIWDKELDTDLKPRLHVTAPFVCKNNPPGQLFVKIAPNLTDDFNADSPQQPRIITYSNFWWKGTLTFTAKMRSSNMWNPIQQHTTTAENIGNYIPTNIGGIKMFPEYSQLIPRKLY

SEQ ID NO: 3 - DNA, 1760 bp, Porcine parvovirus
ggatccgccaccatgtccgagaacgtggagcagcacaacccgataaacgcaggcacagagctgtcggcgactggcaatgagagcggaggcggaggcggcggaggaggtggacgcggcgcaggcggagtgggcgtttcgaccggaagcttcaataatcaaaccgagtttcagtacctgggcgagggtttggtgcggattacggctcacgcgtcccgactgatacatctcaatatgccggagcatgagacctacaagcgtatccatgtcctgaactcggaatcgggcgtcgccggtcagatggtccaagatgatgctcatactcagatggtgacaccctggagcttgatagatgccaacgcatggggcgtgtggttcaaccctgcggattggcagctgataagcaataacatgacagaaatcaatttggttagtttcgagcaagagatatttaatgtcgtgctgaaaaccatcacagagagcgccacgagccccccgacgaagatttacaataacgacctgacggcgtccttgatggtcgccttggacacaaataacaccctcccgtacacccccgcggccccccgcagcgagaccctgggcttttatccctggctgcccaccaagccaacgcagtatcgctactacctgagttgtacacgaaatttgaatccgccgacatacactggtcagtcggagcagatcacggacagcattcaaacgggcctgcactccgatatcatgttttacacgatagagaacgcagtacccatccacctgctgcgtacgggagatgagttctcgaccggtatctatcattttgacacaaaacccttgaaattgacgcacagttggcaaaccaatcgctcgctgggcttgcccccaaagttgttgacggaacccaccaccgagggtgaccaacacccaggcactctccccgcagcaaatacccgcaagggctatcatcaaacgatcaacaatagctataccgaggctaccgccattcggccagcacaggtgggatacaacacaccttacatgaactttgaatactccaacggcggcccgttcctgaccccgatagttccgaccgccgacactcagtacaacgatgacgagccgaacggcgccatcaggtttaccatgggctatcagcacggtcaattgacaacttcgtcgcaagaactggaacgctatacattcaaccctcagagtaagtgtggccgggcacccaaacaacagttcaaccagcaatccccactgaacctgcagaataccaacaatggcacgctgctgccatccgatcccattggaggaaagaccaacatgcatttcatgaacacgctgaatacatacggaccactgaccgccctgaacaataccgcacccgtcttccctaatggccagatctgggataaagagctggatacggacctgaagccccgactccacgtgactgcgccctttgtgtgcaaaaataacccaccgggacagttgttcgtcaaaatagcccccaacttgaccgacgacttcaatgcagacagccctcagcagccgcgaatcatcacctattcgaacttctggtggaagggcacgctgactttcacggctaagatgcgctcgagcaatatgtggaacccaatccagcaacataccacaaccgctgaaaatattggcaattacatccctacgaatataggcggaataaagatgtttccggagtattcccagctcattccacgcaagctgtattaagcggccgc

SEQ ID NO: 4 - DNA, 1760 bp, Porcine parvovirus
ggatccgccaccatgtccgagaacgtggagcagcacaacccgataaacgcaggcacagagctgtcggcgactggcaatgaatcgatcggcggaggcggcggaggaggtggacgcggatcgatcggagtgggcgtttcgaccggaagcttcaataatcaaaccgagtttcagtacctgggcgagggtttggtgcggattacggctcacgcgtcccgactgatacatctcaatatgccggagcatgagacctacaagcgtatccatgtcctgaactcggaatcgggcgtcgccggtcagatggtccaagatgatgctcatactcagatggtgacaccctggagcttgatagatgccaacgcatggggcgtgtggttcaaccctgcggattggcagctgataagcaataacatgacagaaatcaatttggttagtttcgagcaagagatatttaatgtcgtgctgaaaaccatcacagagagcgccacgagccccccgacgaagatttacaataacgacctgacggcgtccttgatggtcgccttggacacaaataacaccctcccgtacacccccgcggccccccgcagcgagaccctgggcttttatccctggctgcccaccaagccaacgcagtatcgctactacctgagttgtacacgaaatttgaatccgccgacatacactggtcagtcggagcagatcacggacagcattcaaacgggcctgcactccgatatcatgttttacacgatagagaacgcagtacccatccacctgctgcgtacgggagatgagttctcgaccggtatctatcattttgacacaaaacccttgaaattgacgcacagttggcaaaccaatcgctcgctgggcttgcccccaaagttgttgacggaacccaccaccgagggtgaccaacacccaggcactctccccgcagcaaatacccgcaagggctatcatcaaacgatcaacaatagctataccgaggctaccgccattcggccagcacaggtgggatacaacacaccttacatgaactttgaatactccaacggcggcccgttcctgaccccgatagttccgaccgccgacactcagtacaacgatgacgagccgaacggcgccatcaggtttaccatgggctatcagcacggtcaattgacaacttcgtcgcaagaactggaacgctatacattcaaccctcagagtaagtgtggccgggcacccaaacaacagttcaaccagcaatccccactgaacctgcagaataccaacaatggcacgctgctgccatccgatcccattggaggaaagaccaacatgcatttcatgaacacgctgaatacatacggaccactgaccgccctgaacaataccgcacccgtcttccctaatggccagatctgggataaagagctggatacggacctgaagccccgactccacgtgactgcgccctttgtgtgcaaaaataacccaccgggacagttgttcgtcaaaatagcccccaacttgaccgacgacttcaatgcagacagccctcagcagccgcgaatcatcacctattcgaacttctggtggaagggcacgctgactttcacggctaagatgcgctcgagcaatatgtggaacccaatccagcaacataccacaaccgctgaaaatattggcaattacatccctacgaatataggcggaataaagatgtttccggagtattcccagctcattccacgcaagctgtattaagcggccgc

SEQ ID NO: 5 - protein, 579 aa, Porcine parvovirus
MSENVEQHNPINAGTELSATGNESIGGGGGGGGRGSIGVGVSTGSFNNQTEFQYLGEGLVRITAHASRLIHLNMPEHETYKRIHVLNSESGVAGQMVQDDAHTQMVTPWSLIDANAWGVWFNPADWQLISNNMTEINLVSFEQAIFNVVLKTITESATSPPTKIYNNDLTASLMVALDTNNTLPYTPAAPRSETLGFYPWLPTKPTQYRYYLSCIRNLNPPTYTGQSEQITDSIQTGLHSDIMFYTIENAVPIHLLRTGDEFSTGIYHFDTKPLKLTHSWQTNRSLGLPPKLLTEPTTEGDQHPGTLPAANTRKGYHQTTNNSYTEATAIRPAQVGYNTPYMNFEYSNGGPFLTPIVPTADTQYNDDEPNGAIRFTMDYQHGQLTTSSQELERYTFNPQSKCGRAPKQQFNQQSPLNLQNTNNGTLLPSDPIGGKTNMHFMNTLNTYGPLTALNNTAPVFPNGQIWDKELDTDLKPRLHVTAPFVCKNNPPGQLFVKIAPNLTDDFNADSPQQPRIITYSNFWWKGTLTFTAKMRSSNMWNPIQQHTTTAENIGNYIPTNIGGIRMFPEYSQLIPRKLY

SEQ ID NO: 6 - protein, 579 aa, Porcine parvovirus; identical to SEQ ID NO: 2

SEQ ID NO: 7 - protein, 579 aa, Porcine parvovirus
MSENVEQHNPINAGTELSATGNESIGGGGGGGGRGSIGVGVSTGSFNNQTEFQYLGEGLVRITAHASRLIHLNMPEHETYKRIHVLNSESGVAGQMVQDDAHTQMVTPWSLIDANAWGVWFNPADWQLISNNMTEINLVSFEQEIFNVVLKTITESATSPPTKIYNNDLTASLMVALDTNNTLPYTPAAPRSETLGFYPWLPTKPTQYRYYLSCTRNLNPPTYTGQSEQITDSIQTGLHSDIMFYTIENAVPIHLLRTGDEFSTGIYHFDTKPLKLTHSWQTNRSLGLPPKLLTEPTTEGDQHPGTLPAANTRKGYHQTINNSYTEATAIRPAQVGYNTPYMNFEYSNGGPFFIPIVPTADTQYNDDEPNGGIRFTMGYQHGQLITSSQEVERYTFNPQRKCGRGAKQQFNQQSPLNIQNTNNGTILPSDPIGGKTNMHFMNTPNTYGPLTAVNNTAPVFPNGQIWDKELDTDLKPRLHVTAPFVCKNNPPGQLFVKIAPNLTDDFNADSPQQPRIITYSNFWWKGTLTFTAKMRSSNMWNPIQQHTTTAENIGNYIPTNIGGIKMFPEYSQLIPRKLY

SEQ ID NO: 8 - protein, 579 aa, Porcine parvovirus
MSENVEQHNPINAGTELSATGNESIGGGGGGGGRGSIGVGVSTGSFNNQTEFQYLGEGLVRITAHASRLIHLNMPEHETYKRIHVLNSESGVAGQMVQDDAHTQMVTPWSLIDANAWGVWFNPADWQLISNNMTEINLVSFEQAIFNVVLKTITESATSPPTKIYNNDLTASLMVALHTNNTLPYTPAAPRSETLGFYPWLPTKPTQYRYYLSCIRNLNPPTYTGQSEQITDSIQTGLHSDIMFYTIENAVPIHLLRTGDEFSTGIYHFDTKPLKLTHSWQTNRSLGLPPKLLTEPTTEGDQHPGTLPAANTRKGYHQTINNSYTEATAIRPAQVGYNTPYMNFEYSNGGPFLTPIVPTADTQYNDDEPNGAIRFTMDYQHGHLTTSSQELERYTFNPQSKCGRTPKQQFNQQSPLNLQNTNNGTLLPSDPIGGKTNMHFMNTLNTYGPLTALNNTAPVFPNGQIWDKELDTDLKPRLHVTAPFVCKNNPPGQLFVKIAPNLTDDFNADSPQQPRIITYSNFWWKGTLTFTAKMRSSNMWNPIQQHTTTAENIGKYIPTNIGGIKMFPEYSQLIPRKLY

SEQ ID NO: 9 - protein, 579 aa, Porcine parvovirus
MSENVEQHNPINAGTELSATGNESIGGGGGGGGRGSIGVGVSTGSFNNQTEFQYLGEGLVRITAHASRLIHLNMPEHETYKRIHVLNSESGVAGQMVQDDAHTQMVTPWSLIDANAWGVWFNPADWQLISNNMTEINLVSFEQEIFNVVLKTITESATSPPTKIYNNDLTASLMVALDTNNTLPYTPAAPRSETLGFYPWLPTKPTQYRYYLSCTRNLNPPTYTGQSEQITDSIQTGLHSDIMFYTIENAVPIHLLRTGDEFSTGIYHFDTKPLKLTHSWQTNRSLGLPPKLLTEPTTEGDQHPGTLPAANTRKGYHQTINNSYTEATAIRPAQVGYNTPYMNFEYSNGGPFLTPIVPTADTQYNDDEPNGAIRFTMGYQHGQLTTSSQELERYTFNPQSKCGRAPKQQFNQQSPLNLQNTNNGTLLPSDPIGGKTNMHFMSTLNTYGPLTALNNTAPVFPNGQIWDKELDTDLKPRLHVTAPFVCKNNPPGQLFVKIAPNLTDDFNADSPQQPRIITYSNFWWKGTLTFTAKMRSSNMWNPIQQHTTTAENIGNYIPTNIGGIKMFPEYSQLIPRKLY

SEQ ID NO: 10 - protein, 579 aa, Porcine parvovirus
MSENVEQHNPINAGTELSATGNESIGGGGGGGGRGSIGVGVSTGSFNNQTEFQYLGEGLVRITAHASRLIHLNMPEHETYKRIHVLNSESGVAGQMVQDDAHTQMVTPWSLIDANAWGVWFNPADWQLISNNMTEINLVSFEQEIFNVVLKTITESATSPPTKIYNNDLTASLMVALDTNNTLPYTPAAPRSETLGFYPWLPTKPTQYRYYLSCTRNLNPPTYTGQSEQITDSIQTGLHSDIMFYTIENAVPIHLLRTGDEFSTGIYHFDTKPLKLTHSWQTNRSLGLPPKLLTEPTTEGDQHPGTLPAANTRKGYHQTTNNSYTEATAIRPAQVGYNTPYMNFEYSNGGPFLTPIVPTADTQYNDDEPNGAIRFTMGYQHGQLTTSSQELERYTFNPQSKCGRAPKQQFNQQSPLNLQNTNNGTLLPSDPIGGKTNMHFMNTLNTYGPLTALNNTAPVFPNGQIWDKELDTDLKPRLHVTAPFVCKNNPPGQLFVKIAPNLTDDFNADSPQQPRIITYSNFWWKGTLTFTAKMRSSNMWNPIQQHTTTAENIGNYIPTNIGGIKMFPEYSQLIPRKLY

SEQ ID NO: 11 - protein, 579 aa, Porcine parvovirus
MSENVEQHNPINAGTELSATGNESGGGGGGGGGRGAGGVGVSTGSFNNQTEFQYLGEGLVRITAHASRLIHLNMPEHETYKRIHVLNSESGVAGQMVQDDAHTQMVTPWSLIDANAWGVWFNPADWQLISNNMTEINLVSFEQAIFNVVLKTITESATSPPTKIYNNDLTASLMVALDTNNTLPYTPAAPRSETLGFYPWLPTKPTQYRYYLSCIRNLNPPTYTGQSEQITDSIQTGLHSDIMFYTIENAVPIHLLRTGDEFSTGIYHFDTKPLKLTHSWQTNRSLGLPPKLLTEPTTEGDQHPGTLPAANTRKGYHQTTNNSYTEATAIRPAQVGYNTPYMNFEYSNGGPFLTPIVPTADTQYNDDEPNGAIRFTMDYQHGQLTTSSQELERYTFNPQSKCGRAPKQQFNQQSPLNLQNTNNGTLLPSDPIGGKTNMHFMNTLNTYGPLTALNNTAPVFPNGQIWDKELDTDLKPRLHVTAPFVCKNNPPGQLFVKIAPNLTDDFNADSPQQPRIITYSNFWWKGTLTFTAKMRSSNMWNPIQQHTTTAENIGNYIPTNIGGIRMFPEYSQLIPRKLY

SEQ ID NO: 12 - protein, 579 aa, Porcine parvovirus; identical to SEQ ID NO: 1

SEQ ID NO: 13 - protein, 579 aa, Porcine parvovirus
MSENVEQHNPINAGTELSATGNESGGGGGGGGGRGAGGVGVSTGSFNNQTEFQYLGEGLVRITAHASRLIHLNMPEHETYKRIHVLNSESGVAGQMVQDDAHTQMVTPWSLIDANAWGVWFNPADWQLISNNMTEINLVSFEQEIFNVVLKTITESATSPPTKIYNNDLTASLMVALDTNNTLPYTPAAPRSETLGFYPWLPTKPTQYRYYLSCTRNLNPPTYTGQSEQITDSIQTGLHSDIMFYTIENAVPIHLLRTGDEFSTGIYHFDTKPLKLTHSWQTNRSLGLPPKLLTEPTTEGDQHPGTLPAANTRKGYHQTINNSYTEATAIRPAQVGYNTPYMNFEYSNGGPFFIPIVPTADTQYNDDEPNGGIRFTMGYQHGQLITSSQEVERYTFNPQRKCGRGAKQQFNQQSPLNIQNTNNGTILPSDPIGGKTNMHFMNTPNTYGPLTAVNNTAPVFPNGQIWDKELDTDLKPRLHVTAPFVCKNNPPGQLFVKIAPNLTDDFNADSPQQPRIITYSNFWWKGTLTFTAKMRSSNMWNPIQQHTTTAENIGNYIPTNIGGIKMFPEYSQLIPRKLY

SEQ ID NO: 14 - protein, 579 aa, Porcine parvovirus
MSENVEQHNPINAGTELSATGNESGGGGGGGGGRGAGGVGVSTGSFNNQTEFQYLGEGLVRITAHASRLIHLNMPEHETYKRIHVLNSESGVAGQMVQDDAHTQMVTPWSLIDANAWGVWFNPADWQLISNNMTEINLVSFEQAIFNVVLKTITESATSPPTKIYNNDLTASLMVALHTNNTLPYTPAAPRSETLGFYPWLPTKPTQYRYYLSCIRNLNPPTYTGQSEQITDSIQTGLHSDIMFYTIENAVPIHLLRTGDEFSTGIYHFDTKPLKLTHSWQTNRSLGLPPKLLTEPTTEGDQHPGTLPAANTRKGYHQTINNSYTEATAIRPAQVGYNTPYMNFEYSNGGPFLTPIVPTADTQYNDDEPNGAIRFTMDYQHGHLTTSSQELERYTFNPQSKCGRTPKQQFNQQSPLNLQNTNNGTLLPSDPIGGKTNMHFMNTLNTYGPLTALNNTAPVFPNGQIWDKELDTDLKPRLHVTAPFVCKNNPPGQLFVKIAPNLTDDFNADSPQQPRIITYSNFWWKGTLTFTAKMRSSNMWNPIQQHTTTAENIGKYIPTNIGGIKMFPEYSQLIPRKLY

SEQ ID NO: 15 - protein, 579 aa, Porcine parvovirus
MSENVEQHNPINAGTELSATGNESGGGGGGGGGRGAGGVGVSTGSFNNQTEFQYLGEGLVRITAHASRLIHLNMPEHETYKRIHVLNSESGVAGQMVQDDAHTQMVTPWSLIDANAWGVWFNPADWQLISNNMTEINLVSFEQEIFNVVLKTITESATSPPTKIYNNDLTASLMVALDTNNTLPYTPAAPRSETLGFYPWLPTKPTQYRYYLSCTRNLNPPTYTGQSEQITDSIQTGLHSDIMFYTIENAVPIHLLRTGDEFSTGIYHFDTKPLKLTHSWQTNRSLGLPPKLLTEPTTEGDQHPGTLPAANTRKGYHQTINNSYTEATAIRPAQVGYNTPYMNFEYSNGGPFLTPIVPTADTQYNDDEPNGAIRFTMGYQHGQLTTSSQELERYTFNPQSKCGRAPKQQFNQQSPLNLQNTNNGTLLPSDPIGGKTNMHFMSTLNTYGPLTALNNTAPVFPNGQIWDKELDTDLKPRLHVTAPFVCKNNPPGQLFVKIAPNLTDDFNADSPQQPRIITYSNFWWKGTLTFTAKMRSSNMWNPIQQHTTTAENIGNYIPTNIGGIKMFPEYSQLIPRKLY

SEQ ID NO: 16 - protein, 579 aa, Porcine parvovirus
MSENVEQHNPINAGTELSATGNESGGGGGGGGGRGAGGVGVSTGSFNNQTEFQYLGEGLVRITAHASRLIHLNMPEHETYKRIHVLNSESGVAGQMVQDDAHTQMVTPWSLIDANAWGVWFNPADWQLISNNMTEINLVSFEQEIFNVVLKTITESATSPPTKIYNNDLTASLMVALDTNNTLPYTPAAPRSETLGFYPWLPTKPTQYRYYLSCTRNLNPPTYTGQSEQITDSIQTGLHSDIMFYTIENAVPIHLLRTGDEFSTGIYHFDTKPLKLTHSWQTNRSLGLPPKLLTEPTTEGDQHPGTLPAANTRKGYHQTTNNSYTEATAIRPAQVGYNTPYMNFEYSNGGPFLTPIVPTADTQYNDDEPNGAIRFTMGYQHGQLTTSSQELERYTFNPQSKCGRAPKQQFNQQSPLNLQNTNNGTLLPSDPIGGKTNMHFMNTLNTYGPLTALNNTAPVFPNGQIWDKELDTDLKPRLHVTAPFVCKNNPPGQLFVKIAPNLTDDFNADSPQQPRIITYSNFWWKGTLTFTAKMRSSNMWNPIQQHTTTAENIGNYIPTNIGGIKMFPEYSQLIPRKLY

SEQ ID NO: 17 - DNA, 15111 bp, Porcine reproductive and respiratory syndrome virus
atgatgtgtagggtattccccctacatacacgacacttctagtgtttgtgtaccttggaggcgtgggtacagccccgccccaccccttggcccctgttctagcccaacaggtatccttctctctcggggcgagtgcgccgcctgctgctcccttgcagcgggaaggacctcccgagtatttccggagagcacctgctttacgggatctccaccctttaaccatgtctgggacgttctcccggtgcatgtgcaccccggctgcccgggtattttggaacgccggccaagtcttttgcacacggtgtctcagtgcgcggtctcttctctctccagagcttcaggacactgacctcggtgcagttggcttgttttacaagcctagggacaagcttcactggaaagtccctatcggcatccctcaggtggaatgtactccatccgggtgctgttggctctcagctgttttccctttggcgcgtatgacctccggcaatcacaacttcctccaacgacttgtgaaggttgctgatgttttgtaccgtgacggttgcttggcacctcgacaccttcgtgaactccaagtttacgagcgcggctgcaactggtacccgatcacggggcccgtgcccgggatgggtttgtttgcgaactccatgcacgtatccgaccagccgttccctggtgccacccatgtgttgactaactcgcctttgcctcaacaggcttgtcggcagccgttctgtccatttgaggaggctcattctagcgtgtacaggtggaagaaatttgtggttttcacggactcctccctcaacggtcgatctcgcatgatgtggacgccggaatccgatgattcagccgccctggaggtactaccgcctgagttagaacgtcaggtcgaaatcctcattcggagttttcctgctcatcaccctgtcgacctggccgactgggagctcactgagtcccctgagaacggtttttccttcaacacgtctcattcttgcggtcaccttgtccagaaccccgacgtgtttgatggcaagtgctggctctcctgctttttgggccagtcggtcgaagtgcgctgccatgaggaacatctagctgacgccttcggttaccaaaccaagtggggcgtgcatggtaagtacctccagcgcaggcttcaagttcgcggcattcgtgctgtagtcgatcctgatggtcccattcacgttgaagcgctgtcttgcccccagtcttggatcaggcacctgactctggatgatgatgtcaccccaggattcgttcgcctgacatcccttcgcattgtgccgaacacagagcctaccacttcccggatctttcggtttggagcgcataagtggtatggcgctgccggcaaacgggctcgtgctaagcgtgccgctaaaagtgagaaggattcggctcccacccccaaggttgccctgccggtccccacctgtggaattaccacctactctccaccgacagacgggtcttgtggttggcatgtccttgccgccataatgaaccggatgataaatggtgacttcacgtcccctctgactcagtacaacagaccagaggatgattgggcttctgattatgatcttgttcaggcgattcaatgtctacgactgcctgctaccgtggttcggaatcgcgcctgtcctaacgccaagtaccttataaaacttaacggagttcactgggaggtagaggtgaggtctggaatggctcctcgctccctttctcgtgaatgtgtggttggcgtttgctctgaaggctgtgtcgcaccgccttatccagcagacgggctacctaaacgtgcactcgaggccttggcgtctgcttacagactaccctccgattgtgttagctctggtattgctgactttcttgctaatccacctcctcaggaattctggaccctcgacaaaatgttgacctccccgtcaccagagcggtccggcttctctagtttgtataaattactattagaggttgttccgcaaaaatgcggtgccacggaaggggctttcatctatgctgttgagaggatgttgaaggattgtccgagctccaaacaggccatggcccttctggcaaaaattaaagttccatcctcaaaggccccgtctgtgtccctggacgagtgtttccctacggatgttttagccgacttcgagccagcatctcaggaaaggccccaaagttccggcgctgctgttgtcctgtgttcaccggatgcaaaagagttcgaggaagcagccccggaagaagttcaagagagtggccacaaggccgtccactctgcactccttgccgagggtcctaacaatgagcaggtacaggtggttgccggtgagcaactgaagctcggcggttgtggtttggcagtcgggaatgctcatgaaggtgctctggtctcagctggtctaattaacctggtaggcgggaatttgtccccctcagaccccatgaaagaaaacatgctcaatagccgggaagacgaaccactggatttgtcccaaccagcaccagcttccacaacgacccttgtgagagagcaaacacccgacaacccaggttctgatgccggtgccctccccgtcaccgttcgagaatttgtcccgacggggcctatactctgtcatgttgagcactgcggcacggagtcgggcgacagcagttcgcctttggatctatctgatgcgcaaaccctggaccagcctttaaatctatccctggccgcttggccagtgagggccaccgcgtctgaccctggctgggtccacggtaggcgcgagcctgtctttgtaaagcctcgaaatgctttctctgatggcgattcagcccttcagttcggggagctttctgaatccagctctgtcatcgagtttgaccggacaaaagatgctccggtggttgacgcccctgtcgacttgacgacttcgaacgaggccctctctgtagtcgatcctttcgaatttgccgaactcaagcgcccgcgtttctccgcacaagccttaattgaccgaggcggtccacttgccgatgtccatgcaaaaataaagaaccgggtatatgaacagtgcctccaagcttgtgagcccggtagtcgtgcaaccccagccaccagggagtggctcgacaaaatgtgggatagggtggacatgaaaacttggcgctgcacctcgcagttccaagctggtcgcattcttgcgtccctcaaattcctccctgacatgattcaagacacaccgcctcctgttcccaggaagaaccgagctagtgacaatgccggcctgaagcaactggtggcacagtgggataggaaattgagtgtgaccccccccccaaaaccggttgggccagtgcttgaccagatcgtccctccgcctacggatatccagcaagaagatgtcaccccctccgatgggccaccccatgcgccggattttcctagtcgagtgagcacgggcgggagttggaaaggccttatgctttccggcacccgtctcgcggggtctatcagccagcgccttatgacatgggtttttgaagttttctcccacctcccagcttttatgctcacacttttctcgccgcggggctctatggctccaggtgattggttgtttgcaggtgtcgttttacttgctctcttgctctgtcgttcttacccgatactcggatgccttcccttattgggtgtcttttctggttctttgcggcgtgttcgtctgggtgtttttggttcttggatggcttttgctgtatttttattctcgactccatccaacccagtcggttcttcttgtgaccacgattcgccggagtgtcatgctgagcttttggctcttgagcagcgccaactttgggaacctgtgcgcggccttgtggtcggcccctcaggcctcttatgtgtcattcttggcaagttactcggtgggtcacgttatctctggcatgttctcctacgtttatgcatgcttgcagatttggccctttctcttgtttatgtggtgtcccaggggcgttgtcacaagtgttggggaaagtgtataaggacagctcctgcggaggtggctcttaatgtatttcctttctcgcgcgccacccgtgtctctcttgtatccttgtgtgatcgattccaaacgccaaaaggggttgatcctgtgcacttggcaacgggttggcgcgggtgctggcgtggtgagagccccatccatcaaccacaccaaaagcccatagcttatgccaatttggatgaaaagaaaatgtctgcccaaacggtggttgctgtcccatacgatcccagtcaggctatcaaatgcctgaaagttctgcaggcgggaggggccatcgtggaccagcctacacctgaggtcgttcgtgtgtccgagatccccttctcagccccatttttcccaaaagttccagtcaacccagattgcagggttgtggtagattcggacacttttgtggctgcggttcgctgcggttactcgacagcacaactggttctgggccggggcaactttgccaagttaaatcagaccccccccaggaactctatctccaccaaaacgactggtggggcctcttacacccttgctgtggctcaagtgtctgcgtggactcttgttcatttcatcctcggtctttggttcacatcacctcaagtgtgtggccgaggaaccgctgacccatggtgttcaaatcctttttcatatcctacctatggccccggagttgtgtgctcctctcgactttgtgtgtctgccgacggggtcaccctgccattgttctcagccgtggcacaactctccggtagagaggtggggatttttattttggtgctcgtctccttgactgctttggcccaccgcatggctcttaaggcagacatgttagtggtcttttcggctttttgtgcttacgcctggcccatgagctcctggttaatctgcttctttcctatactcttgaagtgggttacccttcaccctcttactatgctttgggtgcactcattcttggtgttttgtctgccagcagccggcatcctctcactagggataactggccttctttgggcaattggccgctttacccaggttgccggaattattacaccttatgacatccaccagtacacctctgggccacgtggtgcagctgctgtggccacagccccagaaggcacttatatggccgccgtccggagagctgctttaactgggcgaactttaatcttcaccccgtctgcagttggatcccttctcgaaggtgctttcaggactcataaaccctgccttaacaccgtgaatgttgtaggctcttcccttggttccggaggggttttcaccattgatggcagaagaactgtcgtcactgctgcccatgtgttgaacggcgacacagctagagtcaccggcgactcctacaaccgcatgcacactttcaagaccaatggtgattatgcctggtcccatgctgatgactggcagggcgttgcccctgtggtcaaggttgcgaaggggtaccgcggtcgtgcctactggcaaacatcaactggtgtcgaacccggtatcattggggaagggttcgccttctgttttactaactgcggcgattcggggtcacccgtcatctcagaatctggtgatcttattggaatccacaccggttcaaacaaacttggttctggtcttgtgacaacccctgaaggggagacctgcaccatcaaagaaaccaagctctctgacctttccagacattttgcaggcccaagcgttcctcttggggacattaaattgagtccggccatcatccctgatgtaacatccattccgagtgacttggcatcgctcctagcctccgtccctgtagtggaaggcggcctctcgaccgttcaacttttgtgtgtctttttccttctctggcgcatgatgggccatgcctggacacccattgttgccgtgggcttctttttgctgaatgaaattcttccagcagttttggtccgagccgtgttttcttttgcactctttgtgcttgcatgggccaccccctggtctgcacaggtgttgatgattagactcctcacggcatctctcaaccgcaacaagctttctctggcgttctacgcactcgggggtgtcgtcggtttggcagctgaaatcgggacttttgctggcagattgtctgaattgtctcaagctctttcgacatactgcttcttacctagggtccttgctatgaccagttgtgttcccaccatcatcattggtggactccataccctcggtgtgattctgtggttattcaaataccggtgcctccacaacatgctggttggtgatgggagtttttcaagcgccttcttcctacggtattttgcagagggtaatctcagaaaaggtgtttcacagtcctgtggcatgaataacgagtccctaacggctgctttagcttgcaagttgtcacaggctgaccttgattttttgtccagcttaacgaacttcaagtgctttgtatctgcttcaaacatgaaaaatgctgccggccagtacattgaagcagcgtatgccaaggccctgcgccaagagttggcctctctagttcagattgacaaaatgaaaggagttttgtccaagctcgaggcctttgctgaaacagccaccccgtcccttgacataggtgacgtgattgttctgcttgggcaacatcctcacggatccatcctcgatattaatgtggggactgaaaggaaaactgtgtccgtgcaagagacccggagcctaggcggctccaaattcagtgtttgtactgtcgtgtccaacacacccgtggacgccttgaccggcatcccactccagacaccaacccctctttttgagaatggtccgcgtcatcgcagcgaggaagacgatcttaaagtcgagaggatgaagaaacactgtgtatccctcggcttccacaacatcaatggcaaagtttactgcaaaatttgggacaagtctaccggtgacaccttttacacggatgattcccggtacacccaagaccatgcttttcaggacaggtcagccgactacagagacagggactatgagggtgtgcaaaccaccccccaacagggatttgatccaaagtctgaaacccctgttggcactgttgtgatcggcggtattacgtataacaggtatctgatcaaaggtaaggaggttctggtccccaagcctgacaactgccttgaagctgccaagctgtcccttgagcaagctctcgctgggatgggccaaacttgcgaccttacagctgccgaggtggaaaagctaaagcgcatcattagtcaactccaaggtttgaccactgaacaggctttaaactgttagccgccagcggcttgacccgctgtggccgcggcggcctagttgtgactgaaacggcggtaaaaattataaaataccacagcagaactttcaccttaggccctttagacctaaaagtcacttccgaggtggaggtaaagaaatcaactgagcagggccacgctgttgtggcaaacttatgttccggtgtcatcttgatgagacctcacccaccgtcccttgtcgacgttcttctgaaacccggacttgacacaatacccggcattcaaccagggcatggggccgggaatatgggcgtggacggttctatttgggattttgaaaccgcacccacaaaggcagaactcgagttatccaagcaaataatccaagcatgtgaagttaggcgcggggacgccccgaacctccaactcccttacaagctctatcctgttaggggggatcctgagcggcataaaggccgccttatcaataccaggtttggagatttaccttacaaaactcctcaagacaccaagtccgcaatccacgcggcttgttgcctgcaccccaacggggcccccgtgtctgatggtaaatccacactaggtaccactcttcaacatggtttcgagctttatgtccctactgtgccctatagtgtcatggagtaccttgattcacgccctgacaccccttttatgtgtactaaacatggcacttccaaggctgctgcagaggacctccaaaaatacgacctatccacccaaggatttgtcctgcctggggtcctacgcctagtacgcagattcatctttggccatattggtaaggcgccgccattgttcctcccatcaacctatcccgccaagaactctatggcagggatcaatggccagaggttcccaacaaaggacgttcagagcatacctgaaattgatgaaatgtgtgcccgcgctgtcaaggagaattggcaaactgtgacaccttgcaccctcaagaaacagtactgttccaagcccaaaaccaggaccatcctgggcaccaacaactttattgccttggctcacagatcggcgctcagtggtgtcacccaggcattcatgaagaaggcttggaagtccccaattgccttggggaaaaacaaattcaaggagctgcattgcactgtcgccggcaggtgtcttgaggccgacttggcctcctgtgaccgcagcacccccgccattgtaagatggtttgttgccaacctcctgtatgaacttgcaggatgtgaagagtacttgcctagctatgtgcttaattgctgccatgacctcgtggcaacacaggatggtgccttcacaaaacgcggtggcctgtcgtccggggaccccgtcaccagtgtgtccaacaccgtatattcactggtaatttatgcccagcacatggtattgtcggccttgaaaatgggtcatgaaattggtcttaagttcctcgaggaacagctcaagttcgaggacctccttgaaattcagcctatgttggtatactctgatgatcttgtcttgtacgctgaaagacccacatttcccaattaccactggtgggtcgagcaccttgacctgatgctgggtttcagaacggacccaaagaaaaccgtcataactgataaacccagcttcctcggctgcagaattgaggcagggcgacagctagtccccaatcgcgaccgcatcctggctgctcttgcatatcacatgaaggcgcagaacgcctcagagtattatgcgtctgctgccgcaatcctgatggattcatgtgcttgcattgaccatgaccctgagtggtatgaggacctcatctgcggtattgcccggtgcgcccgccaggatggttatagcttcccaggtccggcatttttcatgtccatgtgggagaagctgagaagtcataatgaagggaagaaattccgccactgcggcatctgcgacgccaaagccgactatgcgtccgcctgtgggcttgatttgtgtttgttccattcgcactttcatcaacactgccctgtcactctgagctgcggtcaccatgccggttcaaaggaatgttcgcagtgtcagtcacctgttggggctggcagatcccctcttgatgccgtgctaaaacaaattccatacaaacctcctcgtactgtcatcatgaaggtgggtaataaaacaacggccctcgatccggggaggtaccagtcccgtcgaggtctcgttgcagtcaagaggggtattgcaggcaatgaagttgatctttctgatggggactaccaagtggtgcctcttttgccgacttgcaaagacataaacatggtgaaggtggcttgcaatgtactactcagcaagttcatagtagggccaccaggttccggaaagaccacctggctactgagtcaagtccaggacgatgatgtcatttacacacccacccatcagactatgtttgatatagtcagtgctctcaaagtttgcaggtattccattccaggagcctcaggactccctttcccaccacctgccaggtccgggccgtgggttaggcttattgccagcgggcacgtccctggccgagtatcatacctcgatgaggctggatattgtaatcatctggacattcttagactgctttccaaaacaccccttgtgtgtttgggtgaccttcagcaacttcaccctgtcggctttgattcctactgttatgtgttcgatcagatgcctcagaagcagctgaccactatttacagatttggccctaacatctgcgcagccatccagccttgttacagggagaaacttgaatctaaggctaggaacactagggtggtttttaccacccggcctgtggcctttggtcaggtgctgacaccataccataaagatcgcatcggctctgcgataaccatagattcatcccagggggccacctttgatattgtgacattgcatctaccatcgccaaagtccctaaataaatcccgagcacttgtagccatcactcgggcaagacacgggttgttcatttatgaccctcataaccagctccaggagtttttcaacttaacccctgagcgcactgattgtaaccttgtgttcagccgtggggatgagctggtagttctgaatgcggataatgcagtcacaactgtagcgaaggcccttgagacaggtccatctcgatttcgagtatcagacccgaggtgcaagtctctcttagccgcttgttcggccagtctggaagggagctgtatgccactaccgcaagtggcacataacctggggttttacttttccccggacagtccaacatttgcacctctgccaaaagagttggcgccacattggccagtggttacccaccagaataatcgggcgtggcctgatcgacttgtcgctagtatgcgcccaattgatgcccgctacagcaagccaatggtcggtgcagggtatgtggtcgggccgtccacctttcttggtactcctggtgtggtgtcatactatctcacactatacatcaggggtgagccccaggccttgccagaaacactcgtttcaacagggcgtatagccacagattgtcgggagtatctcgacgcggctgaggaagaggcagcaaaagaactcccccacgcattcattggcgatgtcaaaggtaccacggttggggggtgtcatcacattacatcaaaatacctacctaggtccctgcctaaggactctgttgccgtagttggagtaagttcgcccggcagggctgctaaagccgtgtgcactctcaccgatgtgtacctccccgaactccggccatatctgcaacctgagacggcatcaaaatgctggaaactcaaattagacttcagggacgtccgactaatggtctggaaaggagccaccgcctatttccagttggaagggcttacatggtcggcgctgcccgactatgccaggtttattcagctgcccaaggatgccgttgtatacattgatccgtgtataggaccggcaacagccaaccgtaaggtcgtgcgaaccacagactggcgggccgacctggcagtgacaccgtatgattacggtgcccagaacattttgacaacagcctggttcgaggacctcgggccgcagtggaagattttggggttgcagccctttaggcgagcatttggctttgaaaacactgaggattgggcaatccttgcacgccgtatgaatgacggcaaggactacactgactataactggaactgtgttcgagaacgcccacacgccatctacgggcgtgctcgtgaccatacgtatcattttgcccctggcacagaattgcaggtagagctaggtaaaccccggctgccgcctgggcaagtgccgtgaattcggggtgatgcaatggggtcactgtggagtaaaatcagccagctgttcgtggacgccttcactgagttccttgttagtgtggttgatattgccattttccttgccatactgtttgggttcaccgtcgcaggatggttactggtctttcttctcagagtggtttgctccgcgcttctccgttcgcgctctgccattcactctcccgaactatcgaaggtcctatgaaggcttgttgcccaactgcagaccggatgtcccacaatttgcagtcaagcacccattgggtatgttttggcacatgcgagtttcccacttgattgatgagatggtctctcgtcgcatttaccagaccatggaacattcaggtcaagcggcctggaagcaggtggttggtgaggccactctcacgaagctgtcagggctcgatatagttactcatttccaacacctggccgcagtggaggcggattcttgccgctttctcagctcacgactcgtgatgctaaaaaatcttgccgttggcaatgtgagcctacagtacaacaccacgttggaccgcgttgagctcatcttccccacgccaggtacgaggcccaagttgaccgatttcagacaatggctcatcagtgtgcacgcttccattttttcctctgtggcttcatctgttaccttgttcatagtgctttggcttcgaattccagctctacgctatgtttttggtttccattggcccacggcaacacatcattcgagctgaccatcaactacaccatatgcatgccctgttctaccagtcaagcggctcgccaaaggctcgagcccggtcgtaacatgtggtgcaaaatagggcatgacaggtgtgaggagcgtgaccatgatgagttgttaatgtccatcccgtccgggtacgacaacctcaaacttgagggttattatgcttggctggcttttttgtccttttcctacgcggcccaattccatccggagttgttcgggatagggaatgtgtcgcgcgtcttcgtggacaagcgacaccagttcatttgtgccgagcatgatggacacaattcaaccgtatctaccggacacaacatctccgcattatatgcggcatattaccaccaccaaatagacgggggcaattggttccatttggaatggctgcggccactcttttcttcctggctggtgctcaacatatcatggtttctgaggcgttcgcctgtaagccctgtttctcgacgcatctatcagatattgagaccaacacgaccgcggctgccggtttcatggtccttcaggacatcaattgtttccgacctcacggggtctcagcagcgcaagagaaaatttccttcggaaagtcgtcccaatgtcgtgaagccgtcggtactccccagtacatcacgataacggctaacgtgaccgacgaatcatacttgtacaacgcggacctgctgatgctttctgcgtgccttttctacgcctcagaaatgagcgagaaaggcttcaaagtcatctttgggaatgtctctggcgttgtttctgcttgtgtcaatttcacagattatgtggcccatgtgacccaacatacccagcagcatcatctggtaattgatcacattcggttgctgcatttcctgacaccatctgcaatgaggtgggctacaaccattgcttgtttgttcgccattctcttggcaatatgagatgttctcacaaattggggcgtttcttgactccgcactcttgcttctggtggctttttttgctgtgtaccggcttgtcctggtcctttgccgatggcaacggcgacagctcgacataccaatacatatataacttgacgatatgcgagctgaatgggaccgactggttgtccagccattttggttgggcagtcgagacctttgtgctttacccggttgccactcatatcctctcactgggttttctcacaacaagccatttttttgacgcgctcggtctcggcgctgtatccactgcaggatttgttggcgggcggtacgtactctgcagcgtctacggcgcttgtgctttcgcagcgttcgtatgttttgtcatccgtgctgctaaaaattgcatggcctgccgctatgcccgtacccggtttaccaacttcattgtggacgaccgggggagagttcatcgatggaagtctccaatagtggtagaaaaattgggcaaagccgaagtcgatggcaacctcgtcaccatcaaacatgtcgtcctcgaaggggttaaagctcaacccttgacgaggacttcggctgagcaatgggaggcctagacgatttttgcaacgatcctatcgccgcacaaaagctcgtgctagcctttagcatcacatacacacctataatgatatacgcccttaaggtgtcacgcggccgactcctggggctgttgcacatcctaatatttctgaactgttcctttacattcggatacatgacatatgtgcattttcaatccaccaaccgtgtcgcacttaccctgggggctgttgtcgcccttctgtggggtgtttacagcttcacagagtcatggaagtttatcacttccagatgcagattgtgttgccttggccggcgatacattctggcccctgcccatcacgtagaaagtgctgcaggtctccattcaatctcagcgtctggtaaccgagcatacgctgtgagaaagcccggactaacatcagtgaacggcactctagtaccaggacttcggagcctcgtgctgggcggcaaacgagctgttaaacgaggagtggttaacctcgtcaagtatggccggtaaaaaccagagccagaagaaaaagaaaagtacagctccgatggggaatggccagccagtcaatcaactgtgccagttgctgggtgcaatgataaagtcccagcgccagcaacctaggggaggacaggccaaaaagaaaaagcctgagaagccacattttcccctggctgctgaagatgacatccggcaccacctcacccagactgaacgctccctctgcttgcaatcgatccagacggctttcaatcaaggcgcaggaactgcgtcgctttcatccagcgggaaggtcagttttcaggttgagtttatgctgccggttgctcatacagtgcgcctgattcgcgtgacttctacatccgccagtcagggtgcaagttaatttgacagtcaggtgaatggccgcgattggcgtgtggcctctgagtcacctattcaattagggcgatcacatgggggtcatacttaatcaggcaggaaccatgtgaccgaaattaaaaaaaaaaaaa

SEQ ID NO: 18 - DNA, 15182 bp, Porcine reproductive and respiratory syndrome virus
tttctccacccctttaaccatgtctgggatacttgatcggtgcacgtgtacccccaatgccagggtgtttatggcggagggccaagtctactgcacacgatgcctcagtgcacggtctctccttcccctgaacctccaagtttctgagctcggggtgctaggcctattctacaggcccgaagagccactccggtggacgttgccacgtgcattccccactgttgagtgctcccccgccggggcctgctggctctctgcaatctttccaatcgcacgaatgaccagtggaaacctgaacttccaacaaagaatgatacgggtcgcagctgagctttacagagccggccagctcacccctgcagtcttgaaggctctacaagtttatgaacggggttgccgctggtaccccattgttggacctgcccctggagtggccgtttacgccaattccctacatgtgagtgataaacctttcccgggagcaactcacgtgttgaccaacctgccgctcccgcagagacccaagcctgaagacttttgcccctttgagtgtgctatggctactgtctatgacattggtcatgacgccgtcatgtatgtggccgaaaggaaaatctcctgggcccctcgtggcggggatgaagtgaaatttgaagctgtccccggggagttgaggttgattgcgaaccggctccgcacctccttcccgccccaccacacagtggacatgtctaagttcgccttcacagcccctgggtgtggtgtttctatgcgggttgaacgccaacacggctgccttcccgctgacactgtccctgaaggcaactgctggtggagcttgtttgactcgcttccactggaagttcagaacaaagaaattcgccatgctaaccaatttggctaccagaccaagcatggtgtctctggcaagtacctacagcggaggctgcaagttaatggtctccgagcagtaactgacctaaacggacctatcgtcgtacagtacttctccgttaaggagagttggatccgccatttgaaactggcgggagaacccagctactctgggtttgaggacctcctcagaataagggttgagcctaacacgtcgccattggctgacaaggaagaaaaaattttccggtttggcagtcacaagtggtacggcgctggaaagagagcaagaaaagcacgctcttgtgcgactgccacagtcgctggccgcgctttgtccgttcgtgaaacccggcaggccaaggagcacgaggttgccggcgccaacaaggctgagcacctcaaacactactccccgcctgccgaagggaattgtggttggcattgcatttccgccatcgccaaccggatggtgaattccaaatttgaaaccacccttcccgaaagagtgagacctccagatgactgggctactgacgaggatcttgtgaatgccatccaaatcctcagactccctgcggccttagacaggaacggtgcttgtactagcgccaagtacgtacttaagctggaaggtgagcattggactgtcactgtggcccctgggatgtccccttctttgctccctcttgaatgtgttcagggctgttgtgggcacaagggcggtcttggttccccagatgcagtcgaggtctccggatttgaccctgcctgccttgaccggctggctgaggtgatgcacctgcctagcagtgctatcccagccgctctggccgaaatgtctggcgattccgatcgttcggcttctccggtcaccaccgtgtggactgtttcgcagttctttgcccgtcacagcggagggaatcaccctgatcaagtgcgcttagggaaaattatcagcctttgtcaggtgattgaggactgctgctgttcccagaacaaaaccaaccgggtcaccccggaggaggtcgcagcaaagattgacctgtacctccgtggtgcaacaaatcttgaagaatgcttggccaggcttgagaaagcgcgcccgccacgcgtaatcgacaccttctttgattgggatgttgtgctccctggggttgaggcggcaacccagacgatcaagctgccccaggtcaaccagtgtcgtgctctggtccctgttgtgactcaaaagtccttggacgacaactcggtccccctgaccgccttttcactggctaactactactaccgtgcgcaaggtgacgaagttcgtcaccgtgaaagactaaccgccgtgctctccaagttggaaaaggttgttcgagaagaatatgggctcatgccaaccgagcctggtccacggcccacactgccacgcgggctcgacgaactcaaagaccagatggaggaggacttgctgaagctggctaacgcccagacgacttcggacatgatggcctgggcagtcgagcaggttgacctaaaaacttgggtcaagaactacccgcggtggacaccaccaccccctccgccaaaagttcagcctcgaaaaacgaagcctgtcaagagcttgccggagagaaagcctgtccccgccccgcgcaggaaggttgggtccgattgtggcagcccggtttcattaggcggcgatgtctctaacagttgggaagatttggctgttagtagcccctttgatctcccgaccccacctgagccggcaacaccttcaagtgagctggtgattgtgtcctcaccgcaatgcatcttcaggccggcgacacccttgagtgagccggctccaattcccgcacctcgcggaactgtgtctcgaccggtgacacccttgagtgagccgatccctgtgcccgcaccgcggcgtaagtttcagcaggtgaaaagattgagttcggcggcggcaatcccaccgtaccagaacgagcccctggatttgtctgcttcctcacagactgaacatgaggcctctcccccagcaccgccgcagagcgggggcgttccgggagtagaggggcatgaagctgaggaaaccctgagtgaaatctcggacatgtcgggtaacattaaacctgcgtccgtgtcatcaagcagctccttgtccagcgtgagaatcacacgcccaaaatactcagctcaagccatcatcgactcgggcgggccctgcagtgggcatctccaagaggtaaaggaaacatgccttagtgtcatgcgcgaggcatgtgatgcgactaagcttgatgaccctgctacgcaggaatggctttctcgcatgtgggatcgggtggacatgctgacttggcgcaacacgtctgtttaccaggcgatttgcaccttagatggcaggttaaagttcctcccaaaaatgatactcgagacaccgccgccctatccgtgtgagtttgtgatgatgcctcacacgcctgcaccttccgtaggtgcggagagcgaccttaccattggctcagttgctactgaagatgttccacgcatcctcgagaaaatagaaaatgtcggcgagatggccaaccagggacccttggccttctccgaggataaaccggtagatgaccaacttgtcaacgacccccggatatcgtcgcggaggcctgacgagagcacatcagctccgtccgcaggcacaggtggcgccggctcttttaccgatttgccgccttcagatggcgcggatacggacgggggggggccgtttcggacggcaaaaagaaaagctgaaaggctctttgaccaactgagccgtcaggtttttgacctcgtctcccatctccctgttttcttctcacgccttttctaccctggcggtggttattctccgggtgattggggttttgcagcttttactctattgtgcctctttttatgttacagttacccagcctttggtattgctcccctcttgggtgtgttttctgggtcttctcggcgcgttcgaatgggggtttttggctgctggttggcttttgctgttggtctgttcaagcctgtgtccgacccagtcggcgctgcttgtgagtttgactcgccagagtgtagaaacatccttcattcttttgagcttctcaaaccttgggaccctgttcgcagccttgttgtgggccccgtcggtctcggtcttgccattcttggcaggttactgggcggggcacgctgcatctggcactttttgcttaggcttggcattgttgcagactgtatcttggctggagcttacgtgctttctcaaggtaggtgtaaaaagtgctggggatcttgtataagaactgctcctaatgaggtcgcttttaacgtgtttcctttcacacgtgcgaccaggtcgtcacttatcgacctgtgcgatcggttttgtgcgccaaaaggaatggaccccatttttctcgccactgggtggcgcgggtgctgggccggccgaagccccattgagcaaccctctgaaaaacccatcgcgtttgcccaattggatgaaaagaagattacggctaggactgtggtcgcccagccttatgaccccaaccaagccgtaaagtgcttgcgggtattgcaggcgggtggggcgatggtggctaaggcggtcccaaaagtggttaaggtttccgctgttccattccgagctcccttctttcccactggagtgaaagttgaccctgattgcagggtcgtggttgaccctgacactttcactgcagctctccggtctggctactccaccacaaacctcgtccttggtgtaggggactttgcccagctaaatggattaaaaatcaggcaaatttccaagccttcagggggaggcccacatctcatggctgccctgcatgttgcctgctcgatggctctgcacatgcttgctgggatttatgtgactgcggtgggttcttgcggcaccggcaccaacgacccgtggtgcgctaacccgtttgccgtccctggctacggacctggctctctctgtacgtccagattgtgcatttcccaacacggccttaccctgcccttgtcagcacttgtggcgggattcggtattcaagaaattgccttggtcgttttgatttttgtttccatcggaggcatggctcataggttgagctgtaaggctgacatgctgtgtgttttgcttgcaattgccagctatgtttgggtacctcttacctggttgctttgtgtgtttccttgctggttgcgctgtttttctttgcaccccctcaccatcctatggttggtgtttttcttgatttctgtgaatatgccttcaggaatcttggccatggtgttgttggtttctctttggcttcttggtcgttatactaatgttgctggccttgtcaccccctacgacattcatcattacaccagtggcccccgcggtgttgccgccttggctaccgcaccagatgggacctacttggccgctgtccgccgcgctgcgttgactggccgcaccatgctgtttaccccgtcccagcttgggtctcttcttgagggtgccttcagaactcgaaagccctcactgaacaccgtcaatgtgatcgggtcctccatgggctctggcggggtgtttaccatcgacgggaaagtcaagtgcgtaactgccgcacatgtccttacgggcaattcagctcgggtttccggggtcggcttcaatcaaatgcttgactttgacgtaaagggagatttcgctatcgctgattgcccgaattggcaaggggctgcccccaagacccaattctgcacggatggatggactggccgtgcctattggctaacatcctctggcgtcgaacccggcgtcattggaaaaggattcgccttctgcttcaccgcatgtggcgattccgggtccccagtgatcaccgaggccggtgagcttgtcggcgttcacacgggatcgaataaacaaggggggggcattgttacgcgcccctcaggccagttttgtaatgtggcacccatcaagctaagcgaattaagtgaattctttgctgggcctaaggtcccgctcggtgatgtgaaggtcggcagccacataattaaagacataagcgaggtgccttcagatctttgtgccttgcttgctgccaaacctgaactggaaggaggcctctccaccgtccaacttctttgtgtgttttttctcctgtggagaatgatgggacatgcctggacgcccttggttgctgtgagtttctttattttgaatgaggttctccctgccgtcctggtccggagtgttttctcctttggaatgtttgtgctatcctggctcacgccatggtctgcgcaagttctgatgatcaggcttctgacagcagctcttaacaggaacagatggtcacttgcctttttcagcctcggtgcagtgaccggttttgtcgcagatcttgcggccactcaggggcatccgttgcaggcagtgatgaatttgagcacctatgcattcctgcctcggatgatggttgtgacctcaccagtcccagtgatcacgtgtggtgtcgtgcacctacttgccatcattttgtacttgtttaagtaccgtggcctgcaccatatccttgttggcgatggagtgttctctgcggctttcttcttgagatactttgccgagggaaagttgagggaaggggtgtcgcaatcctgcggaatgaatcatgagtctctgactggtgccctcgctatgagactcaatgacgaggacttggatttccttatgaaatggactgattttaagtgctttgtttctgcgtccaacatgaggaatgcagcgggtcaatttatcgaggctgcctatgctaaagcacttagagtagaactggcccagttggtacaggttgataaagttcgaggtactttggccaaacttgaagcttttgctgataccgtggctcctcaactctcgcccggtgacattgttgtcgctctcggccacacgcctgttggcagtatcttcgacctaaaggttggtagcaccaagcataccctccaagccattgagaccagagtccttgctgggtccaaaatgaccgtggcgcgcgtcgtcgacccgacccccacgcccccacccgcacccgtgcccatccccctcccaccgaaagttctggagaatggccccaacgcttggggggatgaggaccgtttgaataagaagaagaggcgcaggatggaagccctcggcatctatgttatgggcgggaaaaagtaccagaaattttgggacaagaattccggtgatgtgttttatgaggaggtccataataacacagatgagtgggagtgtctcagagttggcgaccctgccgactttgaccctgagaagggaactctgtgtggacatgtcaccattgaaaataaggcttaccatgtttacacctccccatctggtaagaagttcttggtccccgtcaacccagagaatggaagagttcaatgggaagctgcaaagctttccgtggagcaggccctaggtatgatgaatgtcgacggcgaactgactgccaaagaactggagaaactgaaaagaataattgacaaactccagggcctgactaaggagcagtgtttaaactgctagccgccagcgacttgacccgctgtggtcgcggcggcttggttgttactgaaacagcggtaaaaatagtcaaatttcacaaccggaccttcaccctgggacctgtgaatttaaaagtggccagtgaggttgagctaaaagacgcggttgagcacaaccaacacccggttgcgagaccgatcgatggtggagttgtgctcttgcgttccgcggttccttcgcttatagacgtcttgatctccggtgctgatgcatctcccaagttacttgcccatcacgggccgggaaacactgggatcgatggcacgctctgggattttgagtccgaagccactaaagaggaagtcgcactcagtgcgcaaataatacaggcttgtgacattaggcgcggcgacgctcctgaaattggtctcccttacaagctgtaccctgttaggggtaaccctgagcgggtgaaaggagttctgcagaatacaaggtttggagacataccttacaaaacccccagtgacactggaagcccagtgcacgcggctgcctgccttacgcccaacgccactccggtgactgatgggcgctccgtcttggccacgaccatgccccccgggtttgagttatatgtaccgaccataccagcgtctgtccttgattaccttgactctaggcctgactgccctaaacagctgacagagcacggctgcgaagatgccgcactgaaagacctctctaaatatgacttgtccacccaaggctttgttttacctggagttcttcgccttgtgcggaaatacctgtttgcccatgtaggtaagtgcccacccgttcatcggccttctacttaccctgctaagaattctatggctggaataaatgggaacaggttcccaaccaaggacattcagagcgtccctgaaatcgacgttctgtgcgcacaggctgtgcgagaaaactggcaaactgtcaccccttgtactcttaagaaacagtattgcgggaagaagaagactaggaccatactcggcaccaataacttcatcgcactagcccaccgagcagtgttgagtggtgttacccagggcttcatgaaaaaggcgtttaactcgcccatcgccctcggaaagaacaagtttaaggagctacagactccggtcctgggcaggtgccttgaagctgatctcgcatcctgcgatcgatccacgcctgcaattgtccgctggtttgccgccaaccttctttatgaacttgcctgtgctgaagagcatctaccgtcgtacgtgctgaactgctgccacgacttactggtcacgcagtccggcgcagtgactaagagaggtggcctgtcgtctggcgacccgatcacctctgtgtctaacaccatttatagtttggtgatctatgcacagcatatggtgcttagttacttcaaaagtggtcacccccatggccttctgttcttacaagaccagctaaagtttgaggacatgctcaaggttcaacccctgatcgtctattcggacgacctcgtgctgtatgccgagtctcccaccatgccaaactatcactggtgggttgaacatctgaatttgatgctggggtttcagacggacccaaagaagacagcaataacagactcgccatcatttctaggctgtagaataataaatgggcgccagctagtccccaaccgtgacaggatcctcgcggccctcgcctatcacatgaaggcgagtaatgtttctgaatactatgcctcagcggctgcaatactcatggacagctgtgcttgtttggagtatgatcctgaatggtttgaagaacttgtagttggaatagcgcagtgcgcccgcaaggacggctacagttttcccggcacgccgttcttcatgtccatgtgggaaaaactcaggtccaattatgaggggaagaagtcgagagtgtgcgggtactgcggggccccggccccgtacgctactgcctgtggcctcgacgtctgcatttaccacacccacttccaccagcattgtccagtcacaatctggtgtggccatccagcgggttctggttcttgtagtgagtgcaaatcccctgtagggaaaggcacaagccctttagacgaggtgctggaacaagtcccgtataagcccccacggaccgttatcatgcatgtggagcagggtctcaccccccttgatccaggtagataccaaactcgccgcggactagtctctgtcaggcgtggaattaggggaaatgaagttgaactaccagacggtgattatgctagcaccgccttgctccctacctgcaaagagatcaacatggtcgctgtcgcttccaatgtactgcgcagcaggttcatcatcggcccacccggtgctgggaaaacatactggctccttcaacaggtccaggatggtgatgttatttacacaccaactcaccagaccatgcttgacatgattagggctttggggacgtgccggttcaacgtcccggcaggcacaacgctgcaattccccgtcccctcccgcaccggtccgtgggttcgcatcctagccggcggttggtgtcctggcaagaattccttcctagatgaagcagcgtattgcaatcaccttgatgttttgaggcttcttagtaaaactaccctcacctgtctaggagacttcaagcaactccacccagtgggttttgattctcattgctatgtttttgacatcatgcctcaaactcaactgaagaccatctggaggtttggacagaatatctgtgatgccgttcagccagattacagggacaaactcatgtccatggtcaacacaacccgtgtgacctacgtggaaaaacctgtcaggtatgggcaggtcctcaccccctaccacagggaccgagaggacgacgccatcactattgactccagtcaaggcgccacattcgatgtggttacattgcatttgcccactaaagattcactcaacaggcaaagagcccttgttgccatcaccagggcaagacacgctatctttgtgtatgacccacacaggcagctgcagggcttgtttgatcttcctgcaaaaggcacacccgtcaacctcgcagtgcaccgcgacgggcagctgatcgtgctggatagaaataacaaagaatgcacggtcgctcaggctctaggcaacggggataaatttagggccacagataagcgtgttgtagattctctccgcgccatttgtgctgatctagaagggtcgagctctccgctccccaaggtcgcacacaacttgggattttatttctcacctgatttaacacagtttgctaaactcccagtagaacttgcacctcactggcccgtggtgacaacccagaacaatgaaaagtggccagatcggctggttgccagccttcgccctatccataaatacagccgcgcgtgcatcggtgccggctatatggtgggcccttcggtgtttctaggcactcctggggtcgtgtcatactatctcacaaaatttgttaagggcgaggctcaattgcttccggagacggttttcagcaccggccgaattgaggtagactgccgggaatatcttgatgatcgggagcgagaagttgctgcgtccctcccacacgctttcattggcgacgtcaaaggcactaccgttggaggatgtcatcatgtcacctccagatacctcccacgcgtccttcccaaggaatcagttgcggtagtcggggtttcaagccccggaaaagccgcgaaagcattgtgcacactgacagatgtgtacctcccagatcttgacgcctatctccacccggagacccagtccaagtgctggaaaatgatgttggacttcaaagaagttcgactaatggtctggaaagacaaaacagcctatttccaacttgaaggtcgctatttcacctggtatcagcttgccagctatgcctcgtacatccgtgttcctgtcaactctacggtgtacttggacccctgcatgggccccgccctttgcaacaggagagtcgtcgggtccacccactggggggctgacctcgcggtcaccccttatgattacggcgctaaaattatcctgtctagcgcgtaccatggtgaaatgccccccggatacaaaattctggcgtgcgcggagttctcgttggatgacccagttaagtacaaacatacctgggggtttgaatcggatacagcgtatctgtatgagttcaccggaaacggtgaggactgggaggattacaatgatgcgtttcgtgcgcgccaggaagggaaaatttataaggccactgccaccagcttgaagttttattttcccccgggccctgtcattgaaccaactttaggcctgaattgaaatgaaatggggtccatgcaaagccttttttacaaaattggccaactttttgtggatgctttcacggagttcttggtgtccattgttgatatcactatatttttggccattttgtttggcttcaccatcgccggttggctggtggtcttttgcatcagattggtttgctccgcgatactccgtacgcgctctgccattcactctgagcaattacagaagatcttatgaggcctttctttcccagtgccaagtggacattcccacctggggaactaaacatcctttggggatgctttggcaccataaggtgtcaaccctgattgatgaaatggtgtcgcgtcgaatgtaccgcatcatggaaaaagcagggcaggctgcctggaaacaggtggtgagcgaggctacgctgtctcgcattagtagtttggatgtggtggctcattttcagcatctagccgccattgaagccgagacctgtaaatatttggcctcccggctgcccatgctacacaacctgcgcatgacaggttcaaatgtaaccatagtgtataatagcactttgaatcaggtgtttgctatttttccaacccctggttcccggccaaagcttaatgattttcagcaatggttaatagctgtacattcctccatattttcctctgttgcaacttcttgtactctttttgttgtgctgtggttgcgggttccaatactacgtactgcttttggtttccgctggttaggggcaatttttctttcgaactcacagtgaattacacggtgtgtccaccttgcctcacccggcaagcagccgcagagatctacgaacccggtaggtctctttggtgcaggatagggtatgaccgatgtgaggaggatgatcatgacgagctagggtttatggtaccgcctggcctctccagcgaaggccacttgactagtgtttacgcctggttggcgttcttgtccttcagctacacggcccagttccatcccgagatattcgggatagggaatgtgagtcgagtttatgttgacatcaaacatcaactcatctgcgccgaacatgacgggcagaacaccaccttgcctcgtcatgacaacatttcagccgtgtttcagacctattaccaacatcaagtcgacggcggcaattggtttcacctagaatggcttcgtcccttcttttcctcgtggttggttttaaatgtctcttggtttctcaggcgttcgcctgcaaaccatgtttcagttcgagtcttgcagatattaagaccaacaccaccgcagcggcaagctttgctgtcctccaagacatcagttgccttaggcatcgcgactcggcctctgaggcgattcgcaaaatccctcagtgccgtacggcgatagggacacccgtgtatgttaccatcacagccaatgtgacagatgagaattatttacattcttctgatctcctcatgctttcttcttgccttttctatgcttctgagatgagtgaaaagggatttaaggtggtatttggcaatgtgtcaggcatcgtggctgtgtgtgtcaattttaccagctacgtccaacatgtcaaggagtttacccaacgctccctggtggtcgaccatgtgcggttgctccatttcatgacacctgagaccatgaggtgggcaactgttttagcctgtctttttgccattctgttggcaatttgaatgtttaagtatgttggagaaatgcttgaccgcgggctgttactcgcaattgctttctttgtggtgtatcgtgccgttctgttttgctgtgctcgtcaacgccagcaacgacagcagctcccatctacagctgatttacaacttgacgctatgtgagctgaatggcacagattggctagctaacaaatttgattgggcagtggagagttttgtcatctttcccgttttgactcacattgtctcctatggtgccctcactactagccatttccttgacacagtcgctttagtcactgtgtctaccgccgggtttgttcacgggcggtatgtcctaagtagcatctacgcggtctgtgccctggctgcgttgacttgcttcgtcattaggtttgcaaagaattgcatgtcctggcgctacgcgtgtaccagatataccaactttcttctggacactaagggcagactctatcgttggcggtcgcctgtcatcatagagaaaaggggcaaagttgaggtcgaaggtcatctgatcgacctcaaaagagttgtgcttgatggttccgtggcaacccctataaccagagtttcagcggaacaatggggtcgtccttagatgacttctgtcatgatagcacggctccacaaaaggtgcttttggcgttttctattacctacacgccagtgatgatatatgccctaaaggtgagtcgcggccgactgctagggcttctgcaccttttgatcttcctgaattgtgctttcaccttcgggtacatgactttcgcgcactttcagagtacaaataaggtcgcgctcactatgggagcagtagttgcactcctttggggggtgtactcagccatagaaacctggaaattcatcacctccagatgccgtttgtgcttgctaggccgcaagtacattctggcccctgcccaccacgttgaaagtgccgcaggctttcatccgattgcggcaaatgataaccacgcatttgtcgtccggcgtcccggctccactacggtcaacggcacattggtgcccgggttaaaaagcctcgtgttgggtggcagaaaagctgttaaacagggagtggtaaaccttgtcaaatatgccaaataacaacggcaagcagcagaatagaaagaagggggatggccagccagtcaatcagctgtgccagatgctgggtaagatcatcgctcagcaaaaccagtccagaggcaagggaccgggaaagaaaaataagaagaaaaacccggagaagccccattttcctctagcgactgaagatgatgtcagacatcactttacccctagtgagcggcaattgtgtctgtcgtcaatccagaccgcctttaatcaaggcgctgggacttgcaccctgtcagattcagggaggataagttacactgtggagtttagtttgcctacgcatcatactgtgcgcctgattcgcgtcacagcatcaccctcagcatgatgggctggcattcttgaggcatctcagtgtttgaattggaagaatgtgtggtgaatggcactgattgacattgtgcctctaagcactatatt